European Patent Specification EP 4 043 567 B1, published May 8, 2024. Title: METHODS AND COMPOSITIONS FOR THE TREATMENT OF CANCER. Applicant: CHILDREN'S MEDICAL CENTER CORPORATION. The sequence listing filed with the application follows.

SEQUENCE LISTING (33 sequences)

SEQ ID NO: 1 - DNA, 45 bp, Artificial Sequence
  Description of Artificial Sequence: Synthetic oligonucleotide
  Description of Combined DNA/RNA Molecule: Synthetic oligonucleotide
gcgacugguuacccggucguuuugaagaagaucacccuccuuatt

SEQ ID NO: 2 - DNA, 23 bp, Artificial Sequence
  Description of Artificial Sequence: Synthetic oligonucleotide
  Description of Combined DNA/RNA Molecule: Synthetic oligonucleotide
uaaggagggugaucuucuucatt

SEQ ID NO: 3 - DNA, 45 bp, Artificial Sequence
  Description of Artificial Sequence: Synthetic oligonucleotide
  Description of Combined DNA/RNA Molecule: Synthetic oligonucleotide
gcgacugguuacccggucguuuuaaggagggugaucuucuucatt

SEQ ID NO: 4 - DNA, 20 bp, Artificial Sequence
  Description of Artificial Sequence: Synthetic primer
ttcaccaccatggagaaggc

SEQ ID NO: 5 - DNA, 20 bp, Artificial Sequence
  Description of Artificial Sequence: Synthetic primer
ggcatggactgtggtcatga

SEQ ID NO: 6 - DNA, 21 bp, Artificial Sequence
  Description of Artificial Sequence: Synthetic primer
ctggagcagctgaatggaaag

SEQ ID NO: 7 - DNA, 21 bp, Artificial Sequence
  Description of Artificial Sequence: Synthetic primer
cttgaagtccgccctgtaggt

SEQ ID NO: 8 - DNA, 21 bp, Artificial Sequence
  Description of Artificial Sequence: Synthetic primer
tgccttcatttatcccttgaa

SEQ ID NO: 9 - DNA, 24 bp, Artificial Sequence
  Description of Artificial Sequence: Synthetic primer
ttactacattcagccaaaaagcac

SEQ ID NO: 10 - DNA, 18 bp, Artificial Sequence
  Description of Artificial Sequence: Synthetic primer
gctgccgtcattttctgc

SEQ ID NO: 11 - DNA, 18 bp, Artificial Sequence
  Description of Artificial Sequence: Synthetic primer
tctcactggcccgtcatc

SEQ ID NO: 12 - DNA, 22 bp, Artificial Sequence
  Description of Artificial Sequence: Synthetic primer
ggaggttgcagtgccaacgaag

SEQ ID NO: 13 - DNA, 22 bp, Artificial Sequence
  Description of Artificial Sequence: Synthetic primer
tggaagggaggcagggcataac

SEQ ID NO: 14 - DNA, 22 bp, Artificial Sequence
  Description of Artificial Sequence: Synthetic primer
tttgcccagactcgagctcctg

SEQ ID NO: 15 - DNA, 22 bp, Artificial Sequence
  Description of Artificial Sequence: Synthetic primer
gggtgcaggttcgggattcaac

SEQ ID NO: 16 - protein, 29 aa, Artificial Sequence
  Description of Artificial Sequence: Synthetic peptide
AALEALAEALEALAEALEALAEAAAAGGC

SEQ ID NO: 17 - protein, 30 aa, Artificial Sequence
  Description of Artificial Sequence: Synthetic polypeptide
AALAEALAEALAEALAEALAEALAAAAGGC

SEQ ID NO: 18 - protein, 15 aa, Artificial Sequence
  Description of Artificial Sequence: Synthetic peptide
ALEALAEALEALAEA

SEQ ID NO: 19 - protein, 16 aa, Artificial Sequence
  Description of Artificial Sequence: Synthetic peptide
AAVALLPAVLLALLAP

SEQ ID NO: 20 - protein, 11 aa, Artificial Sequence
  Description of Artificial Sequence: Synthetic peptide
AALLPVLLAAP

SEQ ID NO: 21 - protein, 13 aa, Human immunodeficiency virus
GRKKRRQRRRPPQ

SEQ ID NO: 22 - protein, 16 aa, Artificial Sequence
  Description of Artificial Sequence: Synthetic peptide
RQIKIWFQNRRMKWKK

SEQ ID NO: 23 - DNA, 42 bp, Artificial Sequence
  Description of Artificial Sequence: Synthetic oligonucleotide
  Description of Combined DNA/RNA Molecule: Synthetic oligonucleotide
gcgacugguuacccggucguugcuggagaaccucaugcugtt

SEQ ID NO: 24 - DNA, 21 bp, Artificial Sequence
  Description of Artificial Sequence: Synthetic oligonucleotide
  Description of Combined DNA/RNA Molecule: Synthetic oligonucleotide
cagcaugagguucuccagctt

SEQ ID NO: 25 - DNA, 43 bp, Artificial Sequence
  Description of Artificial Sequence: Synthetic oligonucleotide
  Description of Combined DNA/RNA Molecule: Synthetic oligonucleotide
gcgacugguuacccggucguuuggcuacguccaggagcgcatt

SEQ ID NO: 26 - DNA, 21 bp, Artificial Sequence
  Description of Artificial Sequence: Synthetic oligonucleotide
  Description of Combined DNA/RNA Molecule: Synthetic oligonucleotide
ugcgcuccuggacguagcctt

SEQ ID NO: 27 - RNA, 18 nt, Artificial Sequence
  Description of Artificial Sequence: Synthetic oligonucleotide
uggcuacguccaggagcg

SEQ ID NO: 28 - RNA, 18 nt, Artificial Sequence
  Description of Artificial Sequence: Synthetic oligonucleotide
ugcgcuccuggacguagc

SEQ ID NO: 29 - RNA, 19 nt, Artificial Sequence
  Description of Artificial Sequence: Synthetic oligonucleotide
gcuggagaaccucaugcug

SEQ ID NO: 30 - RNA, 19 nt, Artificial Sequence
  Description of Artificial Sequence: Synthetic oligonucleotide
cagcaugagguucuccagc

SEQ ID NO: 31 - RNA, 21 nt, Artificial Sequence
  Description of Artificial Sequence: Synthetic oligonucleotide
ugaagaagaucacccuccuua

SEQ ID NO: 32 - RNA, 21 nt, Artificial Sequence
  Description of Artificial Sequence: Synthetic oligonucleotide
uaaggagggugaucuucuuca

SEQ ID NO: 33 - RNA, 22 nt, Artificial Sequence
  Description of Artificial Sequence: Synthetic oligonucleotide
gcgacugguuacccggucguuu